European Patent Specification EP 3 423 583 B1, published May 24, 2023. Title: Promoter. Applicant: Oxford Genetics Limited. The sequence listing filed with the application follows.

SEQUENCE LISTING (7 sequences)

SEQ ID NO: 1 - DNA, 433 bp, Artificial Sequence
  Synthetic promoter element
cgtgaggctccggtgcccgtcagtgggcagagcgcacatcgcccacagtccccgagaagttggggggaggggtcggcaattgaaccggtgcctagagaaggtggcgcggggtaaactgggaaagtgatgtcgtgtactggctccgcctttttcccgagggtgggggagaaccgtatataagtgcactagtcgccgtgaacgtcaatggaaagtccctattggcgttactatgggaacatacgtcattattgacgtcaatgacggtaaatggcccgcctggcattatgcccagtacatgaccttatgggactttcctacttggcagtacatctacgtattagtcatcgctattaccatgctgatgcggttttggcagtacatcaatgggcgtggatagcggtttgactcacggggatttccaagtctccacccc

SEQ ID NO: 2 - DNA, 172 bp, Artificial Sequence
  Synthetic promoter element
ctaccgggtaggggaggcgcttttcccaaggcagtctggagcatgcgctttagcagccccgctgggcacttggcgctacacaagtggcctctggcctcgcacacattccacatccaccggtaggcgtcaatggaaagtccctattggcgttactatgggaacatacgtcatt

SEQ ID NO: 3 - DNA, 106 bp, Artificial Sequence
  Synthetic promoter element
agtaatcaattacggggtcattagttcatagcccatatatggagttccgcgttacataacttacggtaaatggcccgcctggctgaccgcccaacgacccccgccc

SEQ ID NO: 4 - DNA, 150 bp, Artificial Sequence
  Synthetic promoter element
attgacgtcaatgggagtttgttttggcaccaaaatcaacgggactttccaaaatgtcgtaacaactccgccccattgacgcaaatgggcggtaggcgtgtacggtgggaggtctatataagcagagctggtttagtgaaccgtcagatc

SEQ ID NO: 5 - DNA, 157 bp, Artificial Sequence
  Synthetic promoter element
tgaagttggtggtgaggccctgggcaggttggtatcaaggttacaagacaggtttaaggagaccaatagaaactgggcatgtggagacagagaagactcttgggtttctgataggcactgactctctctgcctattggtctattttcccacccttag

SEQ ID NO: 6 - DNA, 333 bp, Artificial Sequence
  Synthetic promoter element
gcccaggaagtacacgagaagctccgaggattggctgaagtccaacgtctctgattgcggtggctcagagcacccgtatcattttggaggtgagtggctttggttcccggctgaggtggagtgggctgaggactagactgagccctcggacatggaggtggggatggggcagactcatcccattcttgaccaagcccttgttctgctcccttcccaggctctgtgactggggcaacctgcaaggagctggccagccagcctgacgtggacggcttccttgtgggtggtgcttccctcaagcccgaattcgtggacatcatcaacgccaaacaa

SEQ ID NO: 7 - DNA, 155 bp, Artificial Sequence
  Synthetic promoter element
gttgttcgctttgataaacttccaggattcggagacagtattgaagctcaggtacagaaataatttcacctttctttctctttctattcagtgtggcacatctgtaaacgttcactcttcacttagagacatcctcaaccaaatcaccaaaccaa